European Patent Specification EP 3 532 474 B1, published March 27, 2024. Title: 4,5-ANNULATED 1,2,4-TRIAZOLONES. Applicant: Bayer Aktiengesellschat Bayer Pharma Aktiengesellschaft President and Fellows of Harvard College The General Hospital Corporation The Broad Institute Inc. The sequence listing filed with the application follows.

SEQUENCE LISTING (2 sequences)

SEQ ID NO: 1 - DNA, 6129 bp, pACYC_pelB_POR
ggccgcggcaaagccgtttttccataggctccgcccccctgacaagcatcacgaaatctgacgctcaaatcagtggtggcgaaacccgacaggactataaagataccaggcgtttccccctggcggctccctcgtgcgctctcctgttcctgcctttcggtttaccggtgtcattccgctgttatggccgcgtttgtctcattccacgcctgacactcagttccgggtaggcagttcgctccaagctggactgtatgcacgaaccccccgttcagtccgaccgctgcgccttatccggtaactatcgtcttgagtccaacccggaaagacatgcaaaagcaccactggcagcagccactggtaattgatttagaggagttagtcttgaagtcatgcgccggttaaggctaaactgaaaggacaagttttggtgactgcgctcctccaagccagttacctcggttcaaagagttggtagctcagagaaccttcgaaaaaccgccctgcaaggcggttttttcgttttcagagcaagagattacgcgcagaccaaaacgatctcaagaagatcatcttattaatcagataaaatatttctagatttcagtgcaatttatctcttcaaatgtagcacctgaagtcagccccatacgatataagttgtaattctcatgttagtcatgccccgcgcccaccggaaggagctgactgggttgaaggctctcaagggcatcggtcgagatcccggtgcctaatgagtgagctaacttacattaattgcgttgcgctcactgcccgctttccagtcgggaaacctgtcgtgccagctgcattaatgaatcggccaacgcgcggggagaggcggtttgcgtattgggcgccagggtggtttttcttttcaccagtgagacgggcaacagctgattgcccttcaccgcctggccctgagagagttgcagcaagcggtccacgctggtttgccccagcaggcgaaaatcctgtttgatggtggttaacggcgggatataacatgagctgtcttcggtatcgtcgtatcccactaccgagatgtccgcaccaacgcgcagcccggactcggtaatggcgcgcattgcgcccagcgccatctgatcgttggcaaccagcatcgcagtgggaacgatgccctcattcagcatttgcatggtttgttgaaaaccggacatggcactccagtcgccttcccgttccgctatcggctgaatttgattgcgagtgagatatttatgccagccagccagacgcagacgcgccgagacagaacttaatgggcccgctaacagcgcgatttgctggtgacccaatgcgaccagatgctccacgcccagtcgcgtaccgtcttcatgggagaaaataatactgttgatgggtgtctggtcagagacatcaagaaataacgccggaacattagtgcaggcagcttccacagcaatggcatcctggtcatccagcggatagttaatgatcagcccactgacgcgttgcgcgagaagattgtgcaccgccgctttacaggcttcgacgccgcttcgttctaccatcgacaccaccacgctggcacccagttgatcggcgcgagatttaatcgccgcgacaatttgcgacggcgcgtgcagggccagactggaggtggcaacgccaatcagcaacgactgtttgcccgccagttgttgtgccacgcggttgggaatgtaattcagctccgccatcgccgcttccactttttcccgcgttttcgcagaaacgtggctggcctggttcaccacgcgggaaacggtctgataagagacaccggcatactctgcgacatcgtataacgttactggtttcacattcaccaccctgaattgactctcttccgggcgctatcatgccataccgcgaaaggttttgcaccattcgatggtgtcctggcacgacaggtttcccgactggaaagcgggcagtgagcgcaacgcaattaatgtaagttagctcactcattaggcaccccaggctttacactttatgcttccggctcgtataatgtgtggaattgtgagcggataacaatttcacacaggaaacaggatcgatccatcgatgagcttactccccatccccctgttgacaattaatcatcggctcgtataatgtgtggaattgtgagcggataacaatttcacacaggaaacaggatcagcttactccccatccccctgttgacaattaatcatcggctcgtataatgtgtggaattgtgagcggataacaatttcacacaggaaacaggatccatcgatgcttaggaggtcatatgaaatacctgctgccgaccgctgctgctggtctgctgctcctcgctgcccagccggcgatggccatggatatcggaattaattcggatccgatgggagactcccacgtggacaccagctccaccgtgtccgaggcggtggccgaagaagtatctcttttcagcatgacggacatgattctgttttcgctcatcgtgggtctcctaacctactggttcctctttagaaagaaaaaagaagaagtccccgagttcaccaaaattcagacattgacctcctctgtcagagagagcagctttgtggaaaagatgaagaaaacggggaggaacatcatcgtgttctacggctcccagacggggactgcagaggagtttgccaaccgcctgtccaaggacgcccaccgctacgggatgcgaggcatgtcagcggaccctgaggagtatgacctggccgacctgagcagcctgccagagatcgacaacgccctggtggttttctgcatggccacctacggtgagggagaccccaccgacaatgcccaggacttctacgactggctgcaggagacagacgtggatctctctggggtcaagttcgcggtgtttggtcttgggaacaagacctacgagcacttcaatgccatgggcaagtacgtggacaagcggctggagcagctcggcgcccagcgcatctttgagctggggttgggcgacgacgatgggaacttggaggaggacttcatcacctggcgagagcagttctggccggccgtgtgtgaacactttggggtggaagccactggcgaggagtccagcattcgccagtacgagcttgtggtccacaccgacatagatgcggccaaggtgtacatgggggagatgggccggctgaagagctacgagaaccagaagcccccctttgatgccaagaatccgttcctggctgcagtcaccaccaaccggaagctgaaccagggaaccgagcgccacctcatgcacctggaattggacatctcggactccaaaatcaggtatgaatctggggaccacgtggctgtgtacccagccaacgactctgctctcgtcaaccagctgggcaaaatcctgggtgccgacctggacgtcgtcatgtccctgaacaacctggatgaggagtccaacaagaagcacccattcccgtgccctacgtcctaccgcacggccctcacctactacctggacatcaccaacccgccgcgtaccaacgtgctgtacgagctggcgcagtacgcctcggagccctcggagcaggagctgctgcgcaagatggcctcctcctccggcgagggcaaggagctgtacctgagctgggtggtggaggcccggaggcacatcctggccatcctgcaggactgcccgtccctgcggccccccatcgaccacctgtgtgagctgctgccgcgcctgcaggcccgctactactccatcgcctcatcctccaaggtccaccccaactctgtgcacatctgtgcggtggttgtggagtacgagaccaaggccggccgcatcaacaagggcgtggccaccaactggctgcgggccaaggagcctgccggggagaacggcggccgtgcgctggtgcccatgttcgtgcgcaagtcccagttccgcctgcccttcaaggccaccacgcctgtcatcatggtgggccccggcaccggggtggcacccttcataggcttcatccaggagcgggcctggctgcgacagcagggcaaggaggtgggggagacgctgctgtactacggctgccgccgctcagatgaggactacctgtaccgggaggagctggcgcagttccacagggacggtgcgctcacccagctcaacgtggccttctcccgggagcagtcccacaaggtctacgtccagcacctgctaaagcaagaccgagagcacctgtggaagttgatcgaaggcggtgcccacatctacgtctgtggggatgcacggaacatggccagggatgtgcagaacaccttctacgacatcgtggctgagctcggggccatggagcacgcgcaggcggtggactacatcaagaaactgatgaccaagggccgctactccctggacgtgtggagctaggtcgacaagcttgcggccgcactcgagtctggtaaagaaaccgctgctgcgaaatttgaacgccagcacatggactcgtctactagcgcagcttaattaacctaggctgctgccaccgctgagcaataactagcataaccccttggggcctctaaacgggtcttgaggggttttttgctgaaacctcaggcatttgagaagcacacggtcacactgcttccggtagtcaataaaccggtaaaccagcaatagacataagcggctatttaacgaccctgccctgaaccgacgaccgggtcgaatttgctttcgaatttctgccattcatccgcttattatcacttattcaggcgtagcaaccaggcgtttaagggcaccaataactgccttaaaaaaattacgccccgccctgccactcatcgcagtactgttgtaattcattaagcattctgccgacatggaagccatcacaaacggcatgatgaacctgaatcgccagcggcatcagcaccttgtcgccttgcgtataatatttgcccatagtgaaaacgggggcgaagaagttgtccatattggccacgtttaaatcaaaactggtgaaactcacccagggattggctgagacgaaaaacatattctcaataaaccctttagggaaataggccaggttttcaccgtaacacgccacatcttgcgaatatatgtgtagaaactgccggaaatcgtcgtggtattcactccagagcgatgaaaacgtttcagtttgctcatggaaaacggtgtaacaagggtgaacactatcccatatcaccagctcaccgtctttcattgccatacggaactccggatgagcattcatcaggcgggcaagaatgtgaataaaggccggataaaacttgtgcttatttttctttacggtctttaaaaaggccgtaatatccagctgaacggtctggttataggtacattgagcaactgactgaaatgcctcaaaatgttctttacgatgccattgggatatatcaacggtggtatatccagtgatttttttctccattttagcttccttagctcctgaaaatctcgataactcaaaaaatacgcccggtagtgatcttatttcattatggtgaaagttggaacctcttacgtgccgatcaacgtctcattttcgccaaaagttggcccagggcttcccggtatcaacagggacaccaggatttatttattctgcgaagtgatcttccgtcacaggtatttattcggcgcaaagtgcgtcgggtgatgctgccaacttactgatttagtgtatgatggtgtttttgaggtgctccagtggcttctgtttctatcagctgtccctcctgttcagctactgacggggtggtgcgtaacggcaaaagcaccgccggacatcagcgctagcggagtgtatactggcttactatgttggcactgatgagggtgtcagtgaagtgcttcatgtggcaggagaaaaaaggctgcaccggtgcgtcagcagaatatgtgatacaggatatattccgcttcctcgctcactgactcgctacgctcggtcgttcgactgcggcgagcggaaatggcttacgaacggggcggagatttcctggaagatgccaggaagatacttaacagggaagtgagag

SEQ ID NO: 2 - DNA, 6540 bp, pETDuet_delta3_CYP2C19
ttgaagcatttatcagggttattgtctcatgagcggatacatatttgaatgtatttagaaaaataaacaaataggtcatgaccaaaatcccttaacgtgagttttcgttccactgagcgtcagaccccgtagaaaagatcaaaggatcttcttgagatcctttttttctgcgcgtaatctgctgcttgcaaacaaaaaaaccaccgctaccagcggtggtttgtttgccggatcaagagctaccaactctttttccgaaggtaactggcttcagcagagcgcagataccaaatactgtccttctagtgtagccgtagttaggccaccacttcaagaactctgtagcaccgcctacatacctcgctctgctaatcctgttaccagtggctgctgccagtggcgataagtcgtgtcttaccgggttggactcaagacgatagttaccggataaggcgcagcggtcgggctgaacggggggttcgtgcacacagcccagcttggagcgaacgacctacaccgaactgagatacctacagcgtgagctatgagaaagcgccacgcttcccgaagggagaaaggcggacaggtatccggtaagcggcagggtcggaacaggagagcgcacgagggagcttccagggggaaacgcctggtatctttatagtcctgtcgggtttcgccacctctgacttgagcgtcgatttttgtgatgctcgtcaggggggcggagcctatggaaaaacgccagcaacgcggcctttttacggttcctggccttttgctggccttttgctcacatgttctttcctgcgttatcccctgattctgtggataaccgtattaccgcctttgagtgagctgataccgctcgccgcagccgaacgaccgagcgcagcgagtcagtgagcgaggaagcggaagagcgcctgatgcggtattttctccttacgcatctgtgcggtatttcacaccgcaatggtgcactctcagtacaatctgctctgatgccgcatagttaagccagtatacactccgctatcgctacgtgactgggtcatggctgcgccccgacacccgccaacacccgctgacgcgccctgacgggcttgtctgctcccggcatccgcttacagacaagctgtgaccgtctccgggagctgcatgtgtcagaggttttcaccgtcatcaccgaaacgcgcgaggcagctgcggtaaagctcatcagcgtggtcgtgaagcgattcacagatgtctgcctgttcatccgcgtccagctcgttgagtttctccagaagcgttaatgtctggcttctgataaagcgggccatgttaagggcggttttttcctgtttggtcactgatgcctccgtgtaagggggatttctgttcatgggggtaatgataccgatgaaacgagagaggatgctcacgatacgggttactgatgatgaacatgcccggttactggaacgttgtgagggtaaacaactggcggtatggatgcggcgggaccagagaaaaatcactcagggtcaatgccagcgcttcgttaatacagatgtaggtgttccacagggtagccagcagcatcctgcgatgcagatccggaacataatggtgcagggcgctgacttccgcgtttccagactttacgaaacacggaaaccgaagaccattcatgttgttgctcaggtcgcagacgttttgcagcagcagtcgcttcacgttcgctcgcgtatcggtgattcattctgctaaccagtaaggcaaccccgccagcctagccgggtcctcaacgacaggagcacgatcatgctagtcatgccccgcgcccaccggaaggagctgactgggttgaaggctctcaagggcatcggtcgagatcccggtgcctaatgagtgagctaacttacattaattgcgttgcgctcactgcccgctttccagtcgggaaacctgtcgtgccagctgcattaatgaatcggccaacgcgcggggagaggcggtttgcgtattgggcgccagggtggtttttcttttcaccagtgagacgggcaacagctgattgcccttcaccgcctggccctgagagagttgcagcaagcggtccacgctggtttgccccagcaggcgaaaatcctgtttgatggtggttaacggcgggatataacatgagctgtcttcggtatcgtcgtatcccactaccgagatgtccgcaccaacgcgcagcccggactcggtaatggcgcgcattgcgcccagcgccatctgatcgttggcaaccagcatcgcagtgggaacgatgccctcattcagcatttgcatggtttgttgaaaaccggacatggcactccagtcgccttcccgttccgctatcggctgaatttgattgcgagtgagatatttatgccagccagccagacgcagacgcgccgagacagaacttaatgggcccgctaacagcgcgatttgctggtgacccaatgcgaccagatgctccacgcccagtcgcgtaccgtcttcatgggagaaaataatactgttgatgggtgtctggtcagagacatcaagaaataacgccggaacattagtgcaggcagcttccacagcaatggcatcctggtcatccagcggatagttaatgatcagcccactgacgcgttgcgcgagaagattgtgcaccgccgctttacaggcttcgacgccgcttcgttctaccatcgacaccaccacgctggcacccagttgatcggcgcgagatttaatcgccgcgacaatttgcgacggcgcgtgcagggccagactggaggtggcaacgccaatcagcaacgactgtttgcccgccagttgttgtgccacgcggttgggaatgtaattcagctccgccatcgccgcttccactttttcccgcgttttcgcagaaacgtggctggcctggttcaccacgcgggaaacggtctgataagagacaccggcatactctgcgacatcgtataacgttactggtttcacattcaccaccctgaattgactctcttccgggcgctatcatgccataccgcgaaaggttttgcaccattcgatggtgtcctggcacgacaggtttcccgactggaaagcgggcagtgagcgcaacgcaattaatgtaagttagctcactcattaggcaccccaggctttacactttatgcttccggctcgtataatgtgtggaattgtgagcggataacaatttcacacaggaaacaggatcgatccatcgatgagcttactccccatccccctgttgacaattaatcatcggctcgtataatgtgtggaattgtgagcggataacaatttcacacaggaaacaggatcagcttactccccatccccctgttgacaattaatcatcggctcgtataatgtgtggaattgtgagcggataacaatttcacacaggaaacaggatccatcgatgcttaggaggtcatatggctcgacaatcttctggacgaggaaaactccctcctggccccactcctctcccagtgattggaaatatcctacagatagatattaaggatgtcagcaaatccttaaccaatctctcaaaaatctatggccctgtgttcactctgtattttggcctggaacgcatggtggtgctgcatggatatgaagtggtgaaggaagccctgattgatcttggagaggagttttctggaagaggccatttcccactggctgaaagagctaacagaggatttggaatcgttttcagcaatggaaagagatggaaggagatccggcgtttctccctcatgacgctgcggaattttgggatggggaagaggagcattgaggaccgtgttcaagaggaagcccgctgccttgtggaggagttgagaaaaaccaaggcttcaccctgtgatcccactttcatcctgggctgtgctccctgcaatgtgatctgctccattattttccagaaacgtttcgattataaagatcagcaatttcttaacttgatggaaaaattgaatgaaaacatcaggattgtaagcaccccctggatccagatatgcaataattttcccactatcattgattatttcccgggaacccataacaaattacttaaaaaccttgcttttatggaaagtgatattttggagaaagtaaaagaacaccaagaatcgatggacatcaacaaccctcgggactttattgattgcttcctgatcaaaatggagaaggaaaagcaaaaccaacagtctgaattcactattgaaaacttggtaatcactgcagctgacttacttggagctgggacagagacaacaagcacaaccctgagatatgctctccttctcctgctgaagcacccagaggtcacagctaaagtccaggaagagattgaacgtgtcattggcagaaaccggagcccctgcatgcaggacaggggccacatgccctacacagatgctgtggtgcacgaggtccagagatacatcgacctcatccccaccagcctgccccatgcagtgacctgtgacgttaaattcagaaactacctcattcccaagggcacaaccatattaacttccctcacttctgtgctacatgacaacaaagaatttcccaacccagagatgtttgaccctcgtcactttctggatgaaggtggaaattttaagaaaagtaactacttcatgcctttctcagcaggaaaacggatttgtgtgggagagggcctggcccgcatggagctgtttttattcctgaccttcattttacagaactttaacctgaaatctctgattgacccaaaggaccttgacacaactcctgttgtcaatggatttgcttctgtcccgcccttctatcagctgtgcttcattcctgtctgactcgagtctggtaaagaaaccgctgctgcgaaatttgaacgccagcacatggactcgtctactagcgcagcttaattaacctaggctgctgccaccgctgagcaataactagcataaccccttggggcctctaaacgggtcttgaggggttttttgctgaaaggaggaactatatccggattggcgaatgggacgcgccctgtagcggcgcattaagcgcggcgggtgtggtggttacgcgcagcgtgaccgctacacttgccagcgccctagcgcccgctcctttcgctttcttcccttcctttctcgccacgttcgccggctttccccgtcaagctctaaatcgggggctccctttagggttccgatttagtgctttacggcacctcgaccccaaaaaacttgattagggtgatggttcacgtagtgggccatcgccctgatagacggtttttcgccctttgacgttggagtccacgttctttaatagtggactcttgttccaaactggaacaacactcaaccctatctcggtctattcttttgatttataagggattttgccgatttcggcctattggttaaaaaatgagctgatttaacaaaaatttaacgcgaattttaacaaaatattaacgtttacaatttctggcggcacgatggcatgagattatcaaaaaggatcttcacctagatccttttaaattaaaaatgaagttttaaatcaatctaaagtatatatgagtaaacttggtctgacagttaccaatgcttaatcagtgaggcacctatctcagcgatctgtctatttcgttcatccatagttgcctgactccccgtcgtgtagataactacgatacgggagggcttaccatctggccccagtgctgcaatgataccgcgagacccacgctcaccggctccagatttatcagcaataaaccagccagccggaagggccgagcgcagaagtggtcctgcaactttatccgcctccatccagtctattaattgttgccgggaagctagagtaagtagttcgccagttaatagtttgcgcaacgttgttgccattgctacaggcatcgtggtgtcacgctcgtcgtttggtatggcttcattcagctccggttcccaacgatcaaggcgagttacatgatcccccatgttgtgcaaaaaagcggttagctccttcggtcctccgatcgttgtcagaagtaagttggccgcagtgttatcactcatggttatggcagcactgcataattctcttactgtcatgccatccgtaagatgcttttctgtgactggtgagtactcaaccaagtcattctgagaatagtgtatgcggcgaccgagttgctcttgcccggcgtcaatacgggataataccgcgccacatagcagaactttaaaagtgctcatcattggaaaacgttcttcggggcgaaaactctcaaggatcttaccgctgttgagatccagttcgatgtaacccactcgtgcacccaactgatcttcagcatcttttactttcaccagcgtttctgggtgagcaaaaacaggaaggcaaaatgccgcaaaaaagggaataagggcgacacggaaatgttgaatactcatactcttcctttttcaatcatga